European Patent Application EP 4 269 572 A1, published November 1, 2023. Title: 変異型L-ピペコリン酸水酸化酵素及びそれを利用したcis-5-ヒドロキシ- L-ピペコリン酸の製造方法. Applicant: API Corporation. The sequence listing filed with the application follows.

SEQUENCE LISTING (2 sequences)

SEQ ID NO: 1 - DNA, 885 bp, Xenorhabdus doucetiae
atgatgagcgcaaaactgctggcaagcattgaattgaaccaagaacagatcgagcatgatctgaatattgttggtagcgagatcctggacgtggcgtacagcgagtatgcgtgcggcaattggggtaccattaccctgtggaaccacagcggcgatgctggcgaccagacgagccgcgaatacgttggtcaggcccgtccgactgagctgggccagcaattagactgcattaatcagctgatccgtaacaatttcaacatcagcctgatcaagagcgtgcgcatcttccgtagctataacggtggtgcgatctatccgcacattgactacttggaattcaaccaaggttttaagcgcgtgcacctggttctgaaatccgaccgttcatgtctgaatagcgaagagaacacggtttatcacatgctgcctggtgaagtgtggtttgtcgatggtcatagcgcgcactcggcgatgagcctgagccgtgtcggcaagtactcgctggtcctggactttgattctggcgccaaattcgaagatctgtattctgagagccacaccctgtgtgttgataacctggagccggacattatccatgaccgccagccactgccgaccagcctgcgtgatagcctggcacacattgctgagcatgcggatgaattcaatatccaatccattctgttcctggccacccgttttcactttagctacgcagtgagcattcgtgagtacttccaactcctggacgagtgcttttctcgcaacccgtacaagtccgttcgcgagcgttacgaagcgctgaaagacattttggtgcgtagcggttataccagccacaatgtcaatcatttcaacagcttgtccggtgtcacgatcggctaa

SEQ ID NO: 2 - protein, 294 aa, Xenorhabdus doucetiae
MMSAKLLASIELNQEQIEHDLNIVGSEILDVAYSEYACGNWGTITLWNHSGDAGDQTSREYVGQARPTELGQQLDCINQLIRNNFNISLIKSVRIFRSYNGGAIYPHIDYLEFNQGFKRVHLVLKSDRSCLNSEENTVYHMLPGEVWFVDGHSAHSAMSLSRVGKYSLVLDFDSGAKFEDLYSESHTLCVDNLEPDIIHDRQPLPTSLRDSLAHIAEHADEFNIQSILFLATRFHFSYAVSIREYFQLLDECFSRNPYKSVRERYEALKDILVRSGYTSHNVNHFNSLSGVTIG